European Patent Application EP 4 324 849 A1, published February 21, 2024. Title: Humanized anti-Nectin-4 antibodies. Applicant: Emergence Therapeutics AG. Application EP, filed August 18, 2022. The sequence listing filed with the application follows.

SEQUENCE LISTING (19 sequences)

SEQ ID NO: 1 - protein, 510 aa, Nectin-4
  REGION 1..510: note = Nectin-4
MPLSLGAEMWGPEAWLLLLLLLASFTGRCPAGELETSDVVTVVLGQDAKLPCFYRGDSGEQVGQVAWARVDAGEGAQELALLHSKYGLHVSPAYEGRVEQPPPPRNPLDGSVLLRNAVQADEGEYECRVSTFPAGSFQARLRLRVLVPPLPSLNPGPALEEGQGLTLAASCTAEGSPAPSVTWDTEVKGTTSSRSFKHSRSAAVTSEFHLVPSRSMNGQPLTCVVSHPGLLQDQRITHILHVSFLAEASVRGLEDQNLWHIGREGAMLKCLSEGQPPPSYNWTRLDGPLPSGVRVDGDTLGFPPLTTEHSGIYVCHVSNEFSSRDSQVTVDVLDPQEDSGKQVDLVSASVVVVGVIAALLFCLLVVVVVLMSRYHRRKAQQMTQKYEEELTLTRENSIRRLHSHHTDPRSQPEESVGLRAEGHPDSLKDNSSCSVMSEEPEGRSYSTLTTVREIETQTELLSPGSGRAEEEEDQDEGIKQAMNHFVQENGTLRAKPTGNGIYINGRGHLV

SEQ ID NO: 2 - protein, 118 aa, humanized monoclonal antibody
  REGION 1..118: note = variable heavy chain
QVQLVQSGAEVKKPGASVKVSCKASGFTFNSMYIHWVRQAPGQRLEWMGWIYAGTGGTRYSQKFQGRVTITRDTSASTAYMELSSLRSEDTAVYYCAIRSGFVPMDYWGQGTLVTVSS

SEQ ID NO: 3 - protein, 118 aa, humanized monoclonal antibody
  REGION 1..118: note = variable heavy chain
QVQLVQSGAEVKKPGASVKVSCKASGFTFNSMYISWVRQAPGQRLEWMAWIYAGTGGTRYSQKFQGRVTITRDTSASTAYMELSSLRSEDTAVYYCAIRSGFVPMDYWGQGTLVTVSS

SEQ ID NO: 4 - protein, 118 aa, humanized monoclonal antibody
  REGION 1..118: note = variable heavy chain
QVQLVQSGAEVKKPGASVKVSCKASGFTFNSMYISWVRQAPGQRLEWMAWIYAGTGGTRFNQKFTGKVTITRDTSASTAYMELSSLRSEDTAVYYCAIRSGFVPMDYWGQGTLVTVSS

SEQ ID NO: 5 - protein, 118 aa, humanized monoclonal antibody
  REGION 1..118: note = variable heavy chain
QVQLVQSGAEVKKPGASVKVSCKASGFTFNSMYISWVRQAPGQSLEWMAWIYAGTGGTRFNQKFTGKVTITVDTSASTAYMELSSLRSEDTAVYYCAIRSGFVPMDYWGQGTLVTVSS

SEQ ID NO: 6 - protein, 107 aa, humanized monoclonal antibody
  REGION 1..107: note = variable light chain
DIVMTQSPDSLAVSLGERATINCKSSQSVSNDVAWYQQKPGQPPKLLIYYASNRESGVPDRFSGSGSGTDFTLTISSLQAEDVAVYYCQQDYSSPWTFGQGTKLEIK

SEQ ID NO: 7 - protein, 107 aa, humanized monoclonal antibody
  REGION 1..107: note = variable light chain
DIVMTQSPDSLAVSLGERATINCKASQSVSNDVAWYQQKPGQPPKLLIYYASNRESGVPDRFSGSGSGTDFTLTISSLQAEDVAVYYCQQDYSSPWTFGQGTKLEIK

SEQ ID NO: 8 - protein, 107 aa, humanized monoclonal antibody
  REGION 1..107: note = variable light chain
DIVMTQSPDSLAVSLGERATINCKASQSVSNDVAWYQQKPGQPPKLLIYYASNRYTGVPDRFSGSGSGTDFTLTISSLQAEDVAVYYCQQDYSSPWTFGQGTKLEIK

SEQ ID NO: 9 - protein, 107 aa, humanized monoclonal antibody
  REGION 1..107: note = variable light chain
DIVMTQSPDSLAVSLGERATINCKASQSVSNDVAWYQQKPGQSPKLLIYYASNRYTGVPDRFSGSGSGTDFTLTISSLQAEDVAVYYCQQDYSSPWTFGQGTKLEIK

SEQ ID NO: 10 - protein, 5 aa, humanized monoclonal antibody
  REGION 1..5: note = complementarity-determining-region-H1
SMYIH

SEQ ID NO: 11 - protein, 5 aa, humanized monoclonal antibody
  REGION 1..5: note = complementarity-determining-region-H1
SMYIS

SEQ ID NO: 12 - protein, 17 aa, humanized monoclonal antibody
  REGION 1..17: note = complementarity-determining-region-H2
WIYAGTGGTRYSQKFQG

SEQ ID NO: 13 - protein, 17 aa, humanized monoclonal antibody
  REGION 1..17: note = complementarity-determining-region-H2
WIYAGTGGTRFNQKFTG

SEQ ID NO: 14 - protein, 9 aa, humanized monoclonal antibody
  REGION 1..9: note = complementarity-determining-region-H3
RSGFVPMDY

SEQ ID NO: 15 - protein, 11 aa, humanized monoclonal antibody
  REGION 1..11: note = complementarity-determining-region-L1
KSSQSVSNDVA

SEQ ID NO: 16 - protein, 11 aa, humanized monoclonal antibody
  REGION 1..11: note = complementarity-determining-region-L1
KASQSVSNDVA

SEQ ID NO: 17 - protein, 7 aa, humanized monoclonal antibody
  REGION 1..7: note = complementarity-determining-region-L2
YASNRES

SEQ ID NO: 18 - protein, 7 aa, humanized monoclonal antibody
  REGION 1..7: note = complementarity-determining-region-L2
YASNRYT

SEQ ID NO: 19 - protein, 9 aa, humanized monoclonal antibody
  REGION 1..9: note = complementarity-determining-region-L3
QQDYSSPWT